European Patent Specification EP 3 808 371 B1, published November 22, 2023. Title: Novel Artificial Tears Containing Recombinant Human Lysozyme and Recombinant Human EGF. Applicant: SHAANXI HK BIOTECH CO. LTD. The sequence listing filed with the application follows.

SEQUENCE LISTING (6 sequences)

SEQ ID NO: 1 - protein, 130 aa, Human lysozyme
KVFERCELARTLKRLGMDGYRGISLANWMCLAKWESGYNTRATNYNAGDRSTDYGIFQINSRYWCNDGKTPGAVNACHLSCSALLQDNIADAVACAKRVVRDPQGIRAWVAWRNRCQNRDVRQYVQGCGV

SEQ ID NO: 2 - DNA, 411 bp, Artificial Sequence
ctcgagaaaagaaaggtctttgaaaggtgtgagttggccagaactctgaaaagattgggaatggatggctacaggggaatcagcctagcaaactggatgtgtttggccaaatgggagagtggttacaacacacgagctacaaactacaatgctggagacagaagcactgattatgggatatttcagatcaatagccgctactggtgtaatgatggcaaaaccccaggagcagttaatgcctgtcatttatcctgcagtgctttgctgcaagataacatcgctgatgctgtagcttgtgcaaagagggttgtccgtgatccacaaggcattagagcatgggtggcatggagaaatcgttgtcaaaacagagatgtccgtcagtatgttcaaggttgtggagtgtaagaattc

SEQ ID NO: 3 - DNA, 34 bp, Artificial Sequence
gcctcgagaaaagaaaggtctttgaaaggtgtga

SEQ ID NO: 4 - DNA, 28 bp, Artificial Sequence
cggaattcttacactccacaaccttgaa

SEQ ID NO: 5 - protein, 53 aa, Human epidermal growth factor
NSDSECPLSHDGYCLHDGVCMYIEALDKYACNCVVGYIGERCQYRDLKWWELR

SEQ ID NO: 6 - DNA, 182 bp, Human lysozyme
ctcgagaaaagaaactctgactctgaatgtccattgtctcacgacggttactgtttgcacgacggtgtttgtatgtacatcgaagctttggacaagtacgcttgtaactgtgttgttggttacatcggtgaaagatgtcaatacagagacttgaagtggtgggaattgagataagcggccgc